European Patent Application EP 4 488 295 A2, published January 8, 2025. Title: Anti-Adrenomedullin (ADM) Binder for use in therapy or prevention of symptoms of illness. Applicant: AdrenoMed AG. Application EP. The sequence listing filed with the application follows.

SEQUENCE LISTING (23 sequences)

SEQ ID NO: 1 - protein, 52 aa, Homo sapiens
YRQSMNNFQGLRSFGCRFGTCTVQKLAHQIYQFTDKDKDNVAPRSKISPQGY

SEQ ID NO: 2 - protein, 12 aa, Synthetic construct
  MOD_RES 12: note = C-terminal amidation
CAPRSKISPQGY

SEQ ID NO: 3 - protein, 22 aa, Homo sapiens
CTVQKLAHQIYQFTDKDKDNVA

SEQ ID NO: 4 - protein, 21 aa, Homo sapiens
YRQSMNNFQGLRSFGCRFGTC

SEQ ID NO: 5 - protein, 8 aa, Synthetic construct
GYTFSRYW

SEQ ID NO: 6 - protein, 8 aa, Synthetic construct
ILPGSGST

SEQ ID NO: 7 - protein, 11 aa, Synthetic construct
TEGYEYDGFDY

SEQ ID NO: 8 - protein, 11 aa, Synthetic construct
QSIVYSNGNTY

SEQ ID NO: 9 - protein, 9 aa, Synthetic construct
FQGSHIPYT

SEQ ID NO: 10 - protein, 225 aa, Synthetic construct
QVQLQQSGAELMKPGASVKISCKATGYTFSRYWIEWVKQRPGHGLEWIGEILPGSGSTNYNEKFKGKATITADTSSNTAYMQLSSLTSEDSAVYYCTEGYEYDGFDYWGQGTTLTVSSASTKGPSVFPLAPSSKSTSGGTAALGCLVKDYFPEPVTVSWNSGALTSGVHTFPAVLQSSGLYSLSSVVTVPSSSLGTQTYICNVNHKPSNTKVDKRVEPKHHHHHH

SEQ ID NO: 11 - protein, 225 aa, Synthetic construct
QVQLVQSGAEVKKPGSSVKVSCKASGYTFSRYWISWVRQAPGQGLEWMGRILPGSGSTNYAQKFQGRVTITADESTSTAYMELSSLRSEDTAVYYCTEGYEYDGFDYWGQGTTVTVSSASTKGPSVFPLAPSSKSTSGGTAALGCLVKDYFPEPVTVSWNSGALTSGVHTFPAVLQSSGLYSLSSVVTVPSSSLGTQTYICNVNHKPSNTKVDKRVEPKHHHHHH

SEQ ID NO: 12 - protein, 225 aa, Synthetic construct
QVQLVQSGAEVKKPGSSVKVSCKASGYTFSRYWIEWVRQAPGQGLEWMGRILPGSGSTNYAQKFQGRVTITADESTSTAYMELSSLRSEDTAVYYCTEGYEYDGFDYWGQGTTVTVSSASTKGPSVFPLAPSSKSTSGGTAALGCLVKDYFPEPVTVSWNSGALTSGVHTFPAVLQSSGLYSLSSVVTVPSSSLGTQTYICNVNHKPSNTKVDKRVEPKHHHHHH

SEQ ID NO: 13 - protein, 225 aa, Synthetic construct
QVQLVQSGAEVKKPGSSVKVSCKATGYTFSRYWISWVRQAPGQGLEWMGEILPGSGSTNYAQKFQGRVTITADESTSTAYMELSSLRSEDTAVYYCTEGYEYDGFDYWGQGTTVTVSSASTKGPSVFPLAPSSKSTSGGTAALGCLVKDYFPEPVTVSWNSGALTSGVHTFPAVLQSSGLYSLSSVVTVPSSSLGTQTYICNVNHKPSNTKVDKRVEPKHHHHHH

SEQ ID NO: 14 - protein, 225 aa, Synthetic construct
QVQLVQSGAEVKKPGSSVKVSCKATGYTFSRYWIEWVRQAPGQGLEWMGEILPGSGSTNYAQKFQGRVTITADESTSTAYMELSSLRSEDTAVYYCTEGYEYDGFDYWGQGTTVTVSSASTKGPSVFPLAPSSKSTSGGTAALGCLVKDYFPEPVTVSWNSGALTSGVHTFPAVLQSSGLYSLSSVVTVPSSSLGTQTYICNVNHKPSNTKVDKRVEPKHHHHHH

SEQ ID NO: 15 - protein, 219 aa, Synthetic construct
DVLLSQTPLSLPVSLGDQATISCRSSQSIVYSNGNTYLEWYLQKPGQSPKLLIYRVSNRFSGVPDRFSGSGSGTDFTLKISRVEAEDLGVYYCFQGSHIPYTFGGGTKLEIKRTVAAPSVFIFPPSDEQLKSGTASVVCLLNNFYPREAKVQWKVDNALQSGNSQESVTEQDSKDSTYSLSSTLTLSKADYEKHKVYACEVTHQGLSSPVTKSFNRGEC

SEQ ID NO: 16 - protein, 219 aa, Synthetic construct
DVVMTQSPLSLPVTLGQPASISCRSSQSIVYSNGNTYLNWFQQRPGQSPRRLIYRVSNRDSGVPDRFSGSGSGTDFTLKISRVEAEDVGVYYCFQGSHIPYTFGQGTKLEIKRTVAAPSVFIFPPSDEQLKSGTASVVCLLNNFYPREAKVQWKVDNALQSGNSQESVTEQDSKDSTYSLSSTLTLSKADYEKHKVYACEVTHQGLSSPVTKSFNRGEC

SEQ ID NO: 17 - protein, 219 aa, Synthetic construct
DVVMTQSPLSLPVTLGQPASISCRSSQSIVYSNGNTYLEWFQQRPGQSPRRLIYRVSNRDSGVPDRFSGSGSGTDFTLKISRVEAEDVGVYYCFQGSHIPYTFGQGTKLEIKRTVAAPSVFIFPPSDEQLKSGTASVVCLLNNFYPREAKVQWKVDNALQSGNSQESVTEQDSKDSTYSLSSTLTLSKADYEKHKVYACEVTHQGLSSPVTKSFNRGEC

SEQ ID NO: 18 - protein, 19 aa, Mus musculus
YRQSMNQGSRSNGCRFGTC

SEQ ID NO: 19 - protein, 12 aa, Mus musculus
CTFQKLAHQIYQ

SEQ ID NO: 20 - protein, 12 aa, Synthetic construct
  MOD_RES 12: note = C-terminal amidation
CAPRNKISPQGY

SEQ ID NO: 21 - protein, 12 aa, Homo sapiens
CTVQKLAHQIYQ

SEQ ID NO: 22 - protein, 448 aa, Synthetic construct
QVQLVQSGAEVKKPGSSVKVSCKASGYTFSRYWIEWVRQAPGQGLEWIGEILPGSGSTNYNQKFQGRVTITADTSTSTAYMELSSLRSEDTAVYYCTEGYEYDGFDYWGQGTTVTVSSASTKGPSVFPLAPSSKSTSGGTAALGCLVKDYFPEPVTVSWNSGALTSGVHTFPAVLQSSGLYSLSSVVTVPSSSLGTQTYICNVNHKPSNTKVDKKVEPKSCDKTHTCPPCPAPELLGGPSVFLFPPKPKDTLMISRTPEVTCVVVDVSHEDPEVKFNWYVDGVEVHNAKTKPREEQYNSTYRVVSVLTVLHQDWLNGKEYKCKVSNKALPAPIEKTISKAKGQPREPQVYTLPPSRDELTKNQVSLTCLVKGFYPSDIAVEWESNGQPENNYKTTPPVLDSDGSFFLYSKLTVDKSRWQQGNVFSCSVMHEALHNHYTQKSLSLSPGK

SEQ ID NO: 23 - protein, 219 aa, Synthetic construct
DVVLTQSPLSLPVTLGQPASISCRSSQSIVYSNGNTYLEWYLQRPGQSPRLLIYRVSNRFSGVPDRFSGSGSGTDFTLKISRVEAEDVGVYYCFQGSHIPYTFGGGTKLEIKRTVAAPSVFIFPPSDEQLKSGTASVVCLLNNFYPREAKVQWKVDNALQSGNSQESVTEQDSKDSTYSLSSTLTLSKADYEKHKVYACEVTHQGLSSPVTKSFNRGEC